European Patent Application EP 4 141 033 A1, published March 1, 2023. Title: Anti-CD73-Anti-PD-1 Bispecific Antibody and Use thereof. Applicant: Akeso Biopharma, Inc. Application EP21792313.5. The sequence listing filed with the application follows.

SEQUENCE LISTING (100 sequences)

SEQ ID NO: 1 - DNA, 363 bp, Artificial Sequence
  Synthetic Artificial Sequence
gaggtgcagctgcagcagtccggaccagagctggtgaagcctggcgcctccatgcggatgtcttgtaaggcctctggctacagcttcaccggctatacaatgaactgggtgaagcagtctcacggcaagaatctggagtggatcggcctgatcaacccttacaatgccggcaccagctataaccagaagtttaagggcaaggccaccctgacagtggacaagagctcctctaccgcctacatggagctgctgtccctgacatctgaggatagcgccgtgtactattgcgcccggtccgagtacagatatggcggcgactactttgattattggggccagggcaccacactgacagtgagctcc

SEQ ID NO: 2 - protein, 121 aa, Artificial Sequence
  Synthetic Artificial Sequence
EVQLQQSGPELVKPGASMRMSCKASGYSFTGYTMNWVKQSHGKNLEWIGLINPYNAGTSYNQKFKGKATLTVDKSSSTAYMELLSLTSEDSAVYYCARSEYRYGGDYFDYWGQGTTLTVSS

SEQ ID NO: 3 - protein, 8 aa, Artificial Sequence
  Synthetic Artificial Sequence
GYSFTGYT

SEQ ID NO: 4 - protein, 8 aa, Artificial Sequence
  Synthetic Artificial Sequence
INPYNAGT

SEQ ID NO: 5 - protein, 14 aa, Artificial Sequence
  Synthetic Artificial Sequence
ARSEYRYGGDYFDY

SEQ ID NO: 6 - DNA, 339 bp, Artificial Sequence
  Synthetic Artificial Sequence
gacatcgtgatgacccagtctccaagctccctggcaatgagcgtgggacagaaggtgacaatgtcttgtaagtctagccagagcctgctgaactcctctaatcagaagaactacctggcctggtatcagcagaagccaggccagtctcccaagctgctggtgtactttgccagcaccagggagtccggagtgcctgacagattcatcggctccggctctggcacagacttcaccctgacaatcagctccgtgcaggcagaggacctggcagattatttctgccagcagcactacgacaccccttatacatttggcggcggcaccaagctggagatcaag

SEQ ID NO: 7 - protein, 113 aa, Artificial Sequence
  Synthetic Artificial Sequence
DIVMTQSPSSLAMSVGQKVTMSCKSSQSLLNSSNQKNYLAWYQQKPGQSPKLLVYFASTRESGVPDRFIGSGSGTDFTLTISSVQAEDLADYFCQQHYDTPYTFGGGTKLEIK

SEQ ID NO: 8 - protein, 12 aa, Artificial Sequence
  Synthetic Artificial Sequence
QSLLNSSNQKNY

SEQ ID NO: 9 - protein, 3 aa, Artificial Sequence
  Synthetic Artificial Sequence
FAS

SEQ ID NO: 10 - protein, 9 aa, Artificial Sequence
  Synthetic Artificial Sequence
QQHYDTPYT

SEQ ID NO: 11 - protein, 25 aa, Artificial Sequence
  Synthetic Artificial Sequence
EVQLQQSGPELVKPGASMRMSCKAS

SEQ ID NO: 12 - protein, 17 aa, Artificial Sequence
  Synthetic Artificial Sequence
MNWVKQSHGKNLEWIGL

SEQ ID NO: 13 - protein, 38 aa, Artificial Sequence
  Synthetic Artificial Sequence
SYNQKFKGKATLTVDKSSSTAYMELLSLTSEDSAVYYC

SEQ ID NO: 14 - protein, 11 aa, Artificial Sequence
  Synthetic Artificial Sequence
WGQGTTLTVSS

SEQ ID NO: 15 - protein, 26 aa, Artificial Sequence
  Synthetic Artificial Sequence
DIVMTQSPSSLAMSVGQKVTMSCKSS

SEQ ID NO: 16 - protein, 17 aa, Artificial Sequence
  Synthetic Artificial Sequence
LAWYQQKPGQSPKLLVY

SEQ ID NO: 17 - protein, 36 aa, Artificial Sequence
  Synthetic Artificial Sequence
TRESGVPDRFIGSGSGTDFTLTISSVQAEDLADYFC

SEQ ID NO: 18 - protein, 10 aa, Artificial Sequence
  Synthetic Artificial Sequence
FGGGTKLEIK

SEQ ID NO: 19 - DNA, 363 bp, Artificial Sequence
  Synthetic Artificial Sequence
caggtgcagctggtgcagtctggagcagaggtggtgaagccaggagcctctgtgaaggtgagctgtaaggccagcggctactccttcaccggctatacaatgaactgggtgaggcaggcaccaggacagaatctggagtggatcggcctgatcaacccttacaatgccggcacctcttataaccagaagtttcagggcaaggtgaccctgacagtggacaagtccacctctacagcctacatggagctgagctccctgcggagcgaggatacagccgtgtactattgcgcccggtccgagtacagatatggcggcgactactttgattattggggccagggcaccacactgaccgtgtctagc

SEQ ID NO: 20 - protein, 121 aa, Artificial Sequence
  Synthetic Artificial Sequence
QVQLVQSGAEVVKPGASVKVSCKASGYSFTGYTMNWVRQAPGQNLEWIGLINPYNAGTSYNQKFQGKVTLTVDKSTSTAYMELSSLRSEDTAVYYCARSEYRYGGDYFDYWGQGTTLTVSS

SEQ ID NO: 21 - DNA, 339 bp, Artificial Sequence
  Synthetic Artificial Sequence
gacatcgtgatgacccagtccccaagctccctggccgtgtctgtgggagagcgggtgacaatctcctgtaagtctagccagtctctgctgaactcctctaatcagaagaactacctggcctggtatcagcagaagcccggccaggcccctaagctgctgatctacttcgcctctaccagggagagcggagtgccagacagattctctggcagcggctccggcacagacttcaccctgacaatcagctccgtgcaggcagaggacgtggcagattactattgccagcagcactacgataccccctatacatttggcggcggcaccaagctggagatcaag

SEQ ID NO: 22 - protein, 113 aa, Artificial Sequence
  Synthetic Artificial Sequence
DIVMTQSPSSLAVSVGERVTISCKSSQSLLNSSNQKNYLAWYQQKPGQAPKLLIYFASTRESGVPDRFSGSGSGTDFTLTISSVQAEDVADYYCQQHYDTPYTFGGGTKLEIK

SEQ ID NO: 23 - DNA, 339 bp, Artificial Sequence
  Synthetic Artificial Sequence
gacatcgtgatgacccagtccccaagctccctggccgtgtctgtgggagagcgggtgacaatctcctgtaagtctagccagtctctgctgaactcctctaatcagaagaactacctggcctggtatcagcagaagcccggccaggcccctaagctgctgatctacttcgcctctaccagggagagcggagtgccagacagattctctggcagcggctccggcacagacttcaccctgacaatcagctccctgcaggcagaggacgtggccgtgtactattgccagcagcactacgataccccctatacatttggcggcggcaccaagctggagatcaag

SEQ ID NO: 24 - protein, 113 aa, Artificial Sequence
  Synthetic Artificial Sequence
DIVMTQSPSSLAVSVGERVTISCKSSQSLLNSSNQKNYLAWYQQKPGQAPKLLIYFASTRESGVPDRFSGSGSGTDFTLTISSLQAEDVAVYYCQQHYDTPYTFGGGTKLEIK

SEQ ID NO: 25 - DNA, 1356 bp, Artificial Sequence
  Synthetic Artificial Sequence
caggtgcagctggtgcagtctggagcagaggtggtgaagccaggagcctctgtgaaggtgagctgtaaggccagcggctactccttcaccggctatacaatgaactgggtgaggcaggcaccaggacagaatctggagtggatcggcctgatcaacccttacaatgccggcacctcttataaccagaagtttcagggcaaggtgaccctgacagtggacaagtccacctctacagcctacatggagctgagctccctgcggagcgaggatacagccgtgtactattgcgcccggtccgagtacagatatggcggcgactactttgattattggggccagggcaccacactgaccgtgtctagcgcctccacaaaggggcccagcgtgtttcctctcgccccctcctccaaaagcaccagcggaggaaccgctgctctcggatgtctggtgaaggactacttccctgaacccgtcaccgtgagctggaatagcggcgctctgacaagcggagtccatacattccctgctgtgctgcaaagcagcggactctattccctgtccagcgtcgtcacagtgcccagcagcagcctgggcacccagacctacatctgtaacgtcaaccacaagccctccaacaccaaggtggacaagaaagtggagcccaaatcctgcgacaagacacacacctgtcccccctgtcctgctcccgaagctgctggaggccctagcgtcttcctctttcctcccaaacccaaggacaccctcatgatcagcagaacccctgaagtcacctgtgtcgtcgtggatgtcagccatgaggaccccgaggtgaaattcaactggtatgtcgatggcgtcgaggtgcacaacgccaaaaccaagcccagggaggaacagtacaactccacctacagggtggtgtccgtgctgacagtcctccaccaggactggctgaacggcaaggagtacaagtgcaaggtgtccaacaaggctctccctgcccccattgagaagaccatcagcaaggccaaaggccaacccagggagccccaggtctatacactgcctccctccagggacgaactcaccaagaaccaggtgtccctgacctgcctggtcaagggcttttatcccagcgacatcgccgtcgagtgggagtccaacggacagcccgagaataactacaagaccacccctcctgtcctcgactccgacggctccttcttcctgtacagcaagctgaccgtggacaaaagcaggtggcagcagggaaacgtgttctcctgcagcgtgatgcacgaagccctccacaaccactacacccagaaaagcctgtccctgagccccggcaaatga

SEQ ID NO: 26 - protein, 451 aa, Artificial Sequence
  Synthetic Artificial Sequence
QVQLVQSGAEVVKPGASVKVSCKASGYSFTGYTMNWVRQAPGQNLEWIGLINPYNAGTSYNQKFQGKVTLTVDKSTSTAYMELSSLRSEDTAVYYCARSEYRYGGDYFDYWGQGTTLTVSSASTKGPSVFPLAPSSKSTSGGTAALGCLVKDYFPEPVTVSWNSGALTSGVHTFPAVLQSSGLYSLSSVVTVPSSSLGTQTYICNVNHKPSNTKVDKKVEPKSCDKTHTCPPCPAPEAAGGPSVFLFPPKPKDTLMISRTPEVTCVVVDVSHEDPEVKFNWYVDGVEVHNAKTKPREEQYNSTYRVVSVLTVLHQDWLNGKEYKCKVSNKALPAPIEKTISKAKGQPREPQVYTLPPSRDELTKNQVSLTCLVKGFYPSDIAVEWESNGQPENNYKTTPPVLDSDGSFFLYSKLTVDKSRWQQGNVFSCSVMHEALHNHYTQKSLSLSPGK

SEQ ID NO: 27 - DNA, 660 bp, Artificial Sequence
  Synthetic Artificial Sequence
gacatcgtgatgacccagtccccaagctccctggccgtgtctgtgggagagcgggtgacaatctcctgtaagtctagccagtctctgctgaactcctctaatcagaagaactacctggcctggtatcagcagaagcccggccaggcccctaagctgctgatctacttcgcctctaccagggagagcggagtgccagacagattctctggcagcggctccggcacagacttcaccctgacaatcagctccctgcaggcagaggacgtggccgtgtactattgccagcagcactacgataccccctatacatttggcggcggcaccaagctggagatcaagcgtacggtggcagccccatctgtcttcatttttccccctagtgacgagcagctgaaatccggaacagcctctgtggtctgtctgctgaacaatttctaccctcgcgaagccaaggtgcagtggaaagtcgataacgctctgcagagtggcaattcacaggagagcgtgactgaacaggactccaaggattctacctatagtctgagctccactctgaccctgtccaaagcagattacgaaaagcacaaagtgtatgcctgtgaggtcacccaccaggggctgagttctccagtcaccaaatccttcaacagaggcgaatgt

SEQ ID NO: 28 - protein, 220 aa, Artificial Sequence
  Synthetic Artificial Sequence
DIVMTQSPSSLAVSVGERVTISCKSSQSLLNSSNQKNYLAWYQQKPGQAPKLLIYFASTRESGVPDRFSGSGSGTDFTLTISSLQAEDVAVYYCQQHYDTPYTFGGGTKLEIKRTVAAPSVFIFPPSDEQLKSGTASVVCLLNNFYPREAKVQWKVDNALQSGNSQESVTEQDSKDSTYSLSSTLTLSKADYEKHKVYACEVTHQGLSSPVTKSFNRGEC

SEQ ID NO: 29 - DNA, 1356 bp, Artificial Sequence
  Synthetic Artificial Sequence
caggtgcagctggtgcagtctggagcagaggtggtgaagccaggagcctctgtgaaggtgagctgtaaggccagcggctactccttcaccggctatacaatgaactgggtgaggcaggcaccaggacagaatctggagtggatcggcctgatcaacccttacaatgccggcacctcttataaccagaagtttcagggcaaggtgaccctgacagtggacaagtccacctctacagcctacatggagctgagctccctgcggagcgaggatacagccgtgtactattgcgcccggtccgagtacagatatggcggcgactactttgattattggggccagggcaccacactgaccgtgtctagcgcctccacaaaggggcccagcgtgtttcctctcgccccctcctccaaaagcaccagcggaggaaccgctgctctcggatgtctggtgaaggactacttccctgaacccgtcaccgtgagctggaatagcggcgctctgacaagcggagtccatacattccctgctgtgctgcaaagcagcggactctattccctgtccagcgtcgtcacagtgcccagcagcagcctgggcacccagacctacatctgtaacgtcaaccacaagccctccaacaccaaggtggacaagaaagtggagcccaaatcctgcgacaagacacacacctgtcccccctgtcctgctcccgaagctgctggagcccctagcgtcttcctctttcctcccaaacccaaggacaccctcatgatcagcagaacccctgaagtcacctgtgtcgtcgtggatgtcagccatgaggaccccgaggtgaaattcaactggtatgtcgatggcgtcgaggtgcacaacgccaaaaccaagcccagggaggaacagtacaactccacctacagggtggtgtccgtgctgacagtcctccaccaggactggctgaacggcaaggagtacaagtgcaaggtgtccaacaaggctctccctgcccccattgagaagaccatcagcaaggccaaaggccaacccagggagccccaggtctatacactgcctccctccagggacgaactcaccaagaaccaggtgtccctgacctgcctggtcaagggcttttatcccagcgacatcgccgtcgagtgggagtccaacggacagcccgagaataactacaagaccacccctcctgtcctcgactccgacggctccttcttcctgtacagcaagctgaccgtggacaaaagcaggtggcagcagggaaacgtgttctcctgcagcgtgatgcacgaagccctccacaaccactacacccagaaaagcctgtccctgagccccggcaaatga

SEQ ID NO: 30 - protein, 451 aa, Artificial Sequence
  Synthetic Artificial Sequence
QVQLVQSGAEVVKPGASVKVSCKASGYSFTGYTMNWVRQAPGQNLEWIGLINPYNAGTSYNQKFQGKVTLTVDKSTSTAYMELSSLRSEDTAVYYCARSEYRYGGDYFDYWGQGTTLTVSSASTKGPSVFPLAPSSKSTSGGTAALGCLVKDYFPEPVTVSWNSGALTSGVHTFPAVLQSSGLYSLSSVVTVPSSSLGTQTYICNVNHKPSNTKVDKKVEPKSCDKTHTCPPCPAPEAAGAPSVFLFPPKPKDTLMISRTPEVTCVVVDVSHEDPEVKFNWYVDGVEVHNAKTKPREEQYNSTYRVVSVLTVLHQDWLNGKEYKCKVSNKALPAPIEKTISKAKGQPREPQVYTLPPSRDELTKNQVSLTCLVKGFYPSDIAVEWESNGQPENNYKTTPPVLDSDGSFFLYSKLTVDKSRWQQGNVFSCSVMHEALHNHYTQKSLSLSPGK

SEQ ID NO: 31 - protein, 25 aa, Artificial Sequence
  Synthetic Artificial Sequence
QVQLVQSGAEVVKPGASVKVSCKAS

SEQ ID NO: 32 - protein, 17 aa, Artificial Sequence
  Synthetic Artificial Sequence
MNWVRQAPGQNLEWIGL

SEQ ID NO: 33 - protein, 38 aa, Artificial Sequence
  Synthetic Artificial Sequence
SYNQKFQGKVTLTVDKSTSTAYMELSSLRSEDTAVYYC

SEQ ID NO: 34 - protein, 11 aa, Artificial Sequence
  Synthetic Artificial Sequence
WGQGTTLTVSS

SEQ ID NO: 35 - protein, 26 aa, Artificial Sequence
  Synthetic Artificial Sequence
DIVMTQSPSSLAVSVGERVTISCKSS

SEQ ID NO: 36 - protein, 17 aa, Artificial Sequence
  Synthetic Artificial Sequence
LAWYQQKPGQAPKLLIY

SEQ ID NO: 37 - protein, 36 aa, Artificial Sequence
  Synthetic Artificial Sequence
TRESGVPDRFSGSGSGTDFTLTISSVQAEDVADYYC

SEQ ID NO: 38 - protein, 10 aa, Artificial Sequence
  Synthetic Artificial Sequence
FGGGTKLEIK

SEQ ID NO: 39 - protein, 26 aa, Artificial Sequence
  Synthetic Artificial Sequence
DIVMTQSPSSLAVSVGERVTISCKSS

SEQ ID NO: 40 - protein, 17 aa, Artificial Sequence
  Synthetic Artificial Sequence
LAWYQQKPGQAPKLLIY

SEQ ID NO: 41 - protein, 36 aa, Artificial Sequence
  Synthetic Artificial Sequence
TRESGVPDRFSGSGSGTDFTLTISSLQAEDVAVYYC

SEQ ID NO: 42 - protein, 10 aa, Artificial Sequence
  Synthetic Artificial Sequence
FGGGTKLEIK

SEQ ID NO: 43 - DNA, 354 bp, Artificial Sequence
  Synthetic Artificial Sequence
gaggtcaaactggtggagagcggcggcgggctggtgaagcccggcgggtcactgaaactgagctgcgccgcttccggcttcgcctttagctcctacgacatgtcatgggtgaggcagacccctgagaagcgcctggaatgggtcgctactatcagcggaggcgggcgatacacctactatcctgactctgtcaaagggagattcacaattagtcgggataacgccagaaatactctgtatctgcagatgtctagtctgcggtccgaggatacagctctgtactattgtgcaaaccggtacggcgaagcatggtttgcctattggggacagggcaccctggtgacagtctctgcc

SEQ ID NO: 44 - protein, 118 aa, Artificial Sequence
  Synthetic Artificial Sequence
EVKLVESGGGLVKPGGSLKLSCAASGFAFSSYDMSWVRQTPEKRLEWVATISGGGRYTYYPDSVKGRFTISRDNARNTLYLQMSSLRSEDTALYYCANRYGEAWFAYWGQGTLVTVSA

SEQ ID NO: 45 - protein, 8 aa, Artificial Sequence
  Synthetic Artificial Sequence
GFAFSSYD

SEQ ID NO: 46 - protein, 8 aa, Artificial Sequence
  Synthetic Artificial Sequence
ISGGGRYT

SEQ ID NO: 47 - protein, 11 aa, Artificial Sequence
  Synthetic Artificial Sequence
ANRYGEAWFAY

SEQ ID NO: 48 - DNA, 321 bp, Artificial Sequence
  Synthetic Artificial Sequence
gacattaagatgacacagtccccttcctcaatgtacgctagcctgggcgagcgagtgaccttcacatgcaaagcatcccaggacatcaacacatacctgtcttggtttcagcagaagccaggcaaaagccccaagaccctgatctaccgggccaatagactggtggacggggtccccagcagattctccggatctggcagtgggcaggattactccctgaccatcagctccctggagtatgaagacatgggcatctactattgcctgcagtatgatgagttccctctgacctttggagcaggcacaaaactggaactgaag

SEQ ID NO: 49 - protein, 107 aa, Artificial Sequence
  Synthetic Artificial Sequence
DIKMTQSPSSMYASLGERVTFTCKASQDINTYLSWFQQKPGKSPKTLIYRANRLVDGVPSRFSGSGSGQDYSLTISSLEYEDMGIYYCLQYDEFPLTFGAGTKLELK

SEQ ID NO: 50 - protein, 6 aa, Artificial Sequence
  Synthetic Artificial Sequence
QDINTY

SEQ ID NO: 51 - protein, 3 aa, Artificial Sequence
  Synthetic Artificial Sequence
RAN

SEQ ID NO: 52 - protein, 9 aa, Artificial Sequence
  Synthetic Artificial Sequence
LQYDEFPLT

SEQ ID NO: 53 - protein, 25 aa, Artificial Sequence
  Synthetic Artificial Sequence
EVKLVESGGGLVKPGGSLKLSCAAS

SEQ ID NO: 54 - protein, 17 aa, Artificial Sequence
  Synthetic Artificial Sequence
MSWVRQTPEKRLEWVAT

SEQ ID NO: 55 - protein, 38 aa, Artificial Sequence
  Synthetic Artificial Sequence
YYPDSVKGRFTISRDNARNTLYLQMSSLRSEDTALYYC

SEQ ID NO: 56 - protein, 11 aa, Artificial Sequence
  Synthetic Artificial Sequence
WGQGTLVTVSA

SEQ ID NO: 57 - protein, 26 aa, Artificial Sequence
  Synthetic Artificial Sequence
DIKMTQSPSSMYASLGERVTFTCKAS

SEQ ID NO: 58 - protein, 17 aa, Artificial Sequence
  Synthetic Artificial Sequence
LSWFQQKPGKSPKTLIY

SEQ ID NO: 59 - protein, 36 aa, Artificial Sequence
  Synthetic Artificial Sequence
RLVDGVPSRFSGSGSGQDYSLTISSLEYEDMGIYYC

SEQ ID NO: 60 - protein, 10 aa, Artificial Sequence
  Synthetic Artificial Sequence
FGAGTKLELK

SEQ ID NO: 61 - DNA, 354 bp, Artificial Sequence
  Synthetic Artificial Sequence
gaagtgcagctggtcgagtctgggggagggctggtgcagcccggcgggtcactgcgactgagctgcgcagcttccggattcgcctttagctcctacgacatgtcctgggtgcgacaggcaccaggaaagggactggattgggtcgctactatctcaggaggcgggagatacacctactatcctgacagcgtcaagggccggttcacaatctctagagataacagtaagaacaatctgtatctgcagatgaacagcctgagggctgaggacaccgcactgtactattgtgccaaccgctacggggaagcatggtttgcctattgggggcagggaaccctggtgacagtctctagt

SEQ ID NO: 62 - protein, 118 aa, Artificial Sequence
  Synthetic Artificial Sequence
EVQLVESGGGLVQPGGSLRLSCAASGFAFSSYDMSWVRQAPGKGLDWVATISGGGRYTYYPDSVKGRFTISRDNSKNNLYLQMNSLRAEDTALYYCANRYGEAWFAYWGQGTLVTVSS

SEQ ID NO: 63 - DNA, 321 bp, Artificial Sequence
  Synthetic Artificial Sequence
gacattcagatgactcagagcccctcctccatgtccgcctctgtgggcgacagggtcaccttcacatgccgcgctagtcaggatatcaacacctacctgagctggtttcagcagaagccagggaaaagccccaagacactgatctaccgggctaatagactggtgtctggagtcccaagtcggttcagtggctcagggagcggacaggactacactctgaccatcagctccctgcagcctgaggacatggcaacctactattgcctgcagtatgatgagttcccactgacctttggcgccgggacaaaactggagctgaag

SEQ ID NO: 64 - protein, 107 aa, Artificial Sequence
  Synthetic Artificial Sequence
DIQMTQSPSSMSASVGDRVTFTCRASQDINTYLSWFQQKPGKSPKTLIYRANRLVSGVPSRFSGSGSGQDYTLTISSLQPEDMATYYCLQYDEFPLTFGAGTKLELK

SEQ ID NO: 65 - DNA, 1344 bp, Artificial Sequence
  Synthetic Artificial Sequence
gaagtgcagctggtcgagtctgggggagggctggtgcagcccggcgggtcactgcgactgagctgcgcagcttccggattcgcctttagctcctacgacatgtcctgggtgcgacaggcaccaggaaagggactggattgggtcgctactatctcaggaggcgggagatacacctactatcctgacagcgtcaagggccggttcacaatctctagagataacagtaagaacaatctgtatctgcagatgaacagcctgagggctgaggacaccgcactgtactattgtgccaaccgctacggggaagcatggtttgcctattgggggcagggaaccctggtgacagtctctagtgccagcaccaaaggacctagcgtgtttcctctcgccccctcctccaaaagcaccagcggaggaaccgctgctctcggatgtctggtgaaggactacttccctgaacccgtcaccgtgagctggaatagcggcgctctgacaagcggagtccatacattccctgctgtgctgcaaagcagcggactctattccctgtccagcgtcgtcacagtgcccagcagcagcctgggcacccagacctacatctgtaacgtcaaccacaagccctccaacaccaaggtggacaagaaagtggagcccaaatcctgcgacaagacacacacctgtcccccctgtcctgctcccgaactcctcggaggccctagcgtcttcctctttcctcccaaacccaaggacaccctcatgatcagcagaacccctgaagtcacctgtgtcgtcgtggatgtcagccatgaggaccccgaggtgaaattcaactggtatgtcgatggcgtcgaggtgcacaacgccaaaaccaagcccagggaggaacagtacaactccacctacagggtggtgtccgtgctgacagtcctccaccaggactggctgaacggcaaggagtacaagtgcaaggtgtccaacaaggctctccctgcccccattgagaagaccatcagcaaggccaaaggccaacccagggagccccaggtctatacactgcctccctccagggacgaactcaccaagaaccaggtgtccctgacctgcctggtcaagggcttttatcccagcgacatcgccgtcgagtgggagtccaacggacagcccgagaataactacaagaccacccctcctgtcctcgactccgacggctccttcttcctgtacagcaagctgaccgtggacaaaagcaggtggcagcagggaaacgtgttctcctgcagcgtgatgcacgaagccctccacaaccactacacccagaaaagcctgtccctgagccccggcaaa

SEQ ID NO: 66 - protein, 448 aa, Artificial Sequence
  Synthetic Artificial Sequence
EVQLVESGGGLVQPGGSLRLSCAASGFAFSSYDMSWVRQAPGKGLDWVATISGGGRYTYYPDSVKGRFTISRDNSKNNLYLQMNSLRAEDTALYYCANRYGEAWFAYWGQGTLVTVSSASTKGPSVFPLAPSSKSTSGGTAALGCLVKDYFPEPVTVSWNSGALTSGVHTFPAVLQSSGLYSLSSVVTVPSSSLGTQTYICNVNHKPSNTKVDKKVEPKSCDKTHTCPPCPAPELLGGPSVFLFPPKPKDTLMISRTPEVTCVVVDVSHEDPEVKFNWYVDGVEVHNAKTKPREEQYNSTYRVVSVLTVLHQDWLNGKEYKCKVSNKALPAPIEKTISKAKGQPREPQVYTLPPSRDELTKNQVSLTCLVKGFYPSDIAVEWESNGQPENNYKTTPPVLDSDGSFFLYSKLTVDKSRWQQGNVFSCSVMHEALHNHYTQKSLSLSPGK

SEQ ID NO: 67 - DNA, 642 bp, Artificial Sequence
  Synthetic Artificial Sequence
gacattcagatgactcagagcccctcctccatgtccgcctctgtgggcgacagggtcaccttcacatgccgcgctagtcaggatatcaacacctacctgagctggtttcagcagaagccagggaaaagccccaagacactgatctaccgggctaatagactggtgtctggagtcccaagtcggttcagtggctcagggagcggacaggactacactctgaccatcagctccctgcagcctgaggacatggcaacctactattgcctgcagtatgatgagttcccactgacctttggcgccgggacaaaactggagctgaagcgaactgtggccgctccctccgtcttcatttttcccccttctgacgaacagctgaaatcaggcacagccagcgtggtctgtctgctgaacaatttctaccctagagaggcaaaagtgcagtggaaggtcgataacgccctgcagtccggcaacagccaggagagtgtgactgaacaggactcaaaagatagcacctattccctgtctagtacactgactctgtccaaggctgattacgagaagcacaaagtgtatgcatgcgaagtgacacatcagggactgtcaagccccgtgactaagtcttttaaccggggcgaatgt

SEQ ID NO: 68 - protein, 214 aa, Artificial Sequence
  Synthetic Artificial Sequence
DIQMTQSPSSMSASVGDRVTFTCRASQDINTYLSWFQQKPGKSPKTLIYRANRLVSGVPSRFSGSGSGQDYTLTISSLQPEDMATYYCLQYDEFPLTFGAGTKLELKRTVAAPSVFIFPPSDEQLKSGTASVVCLLNNFYPREAKVQWKVDNALQSGNSQESVTEQDSKDSTYSLSSTLTLSKADYEKHKVYACEVTHQGLSSPVTKSFNRGEC

SEQ ID NO: 69 - DNA, 1344 bp, Artificial Sequence
  Synthetic Artificial Sequence
gaagtgcagctggtcgagtctgggggagggctggtgcagcccggcgggtcactgcgactgagctgcgcagcttccggattcgcctttagctcctacgacatgtcctgggtgcgacaggcaccaggaaagggactggattgggtcgctactatctcaggaggcgggagatacacctactatcctgacagcgtcaagggccggttcacaatctctagagataacagtaagaacaatctgtatctgcagatgaacagcctgagggctgaggacaccgcactgtactattgtgccaaccgctacggggaagcatggtttgcctattgggggcagggaaccctggtgacagtctctagtgccagcaccaaagggcccagcgtgtttcctctcgccccctcctccaaaagcaccagcggaggaaccgctgctctcggatgtctggtgaaggactacttccctgaacccgtcaccgtgagctggaatagcggcgctctgacaagcggagtccatacattccctgctgtgctgcaaagcagcggactctattccctgtccagcgtcgtcacagtgcccagcagcagcctgggcacccagacctacatctgtaacgtcaaccacaagccctccaacaccaaggtggacaagaaagtggagcccaaatcctgcgacaagacacacacctgtcccccctgtcctgctcccgaagctgctggagcccctagcgtcttcctctttcctcccaaacccaaggacaccctcatgatcagcagaacccctgaagtcacctgtgtcgtcgtggatgtcagccatgaggaccccgaggtgaaattcaactggtatgtcgatggcgtcgaggtgcacaacgccaaaaccaagcccagggaggaacagtacaactccacctacagggtggtgtccgtgctgacagtcctccaccaggactggctgaacggcaaggagtacaagtgcaaggtgtccaacaaggctctccctgcccccattgagaagaccatcagcaaggccaaaggccaacccagggagccccaggtctatacactgcctccctccagggacgaactcaccaagaaccaggtgtccctgacctgcctggtcaagggcttttatcccagcgacatcgccgtcgagtgggagtccaacggacagcccgagaataactacaagaccacccctcctgtcctcgactccgacggctccttcttcctgtacagcaagctgaccgtggacaaaagcaggtggcagcagggaaacgtgttctcctgcagcgtgatgcacgaagccctccacaaccactacacccagaaaagcctgtccctgagccccggcaaa

SEQ ID NO: 70 - protein, 448 aa, Artificial Sequence
  Synthetic Artificial Sequence
EVQLVESGGGLVQPGGSLRLSCAASGFAFSSYDMSWVRQAPGKGLDWVATISGGGRYTYYPDSVKGRFTISRDNSKNNLYLQMNSLRAEDTALYYCANRYGEAWFAYWGQGTLVTVSSASTKGPSVFPLAPSSKSTSGGTAALGCLVKDYFPEPVTVSWNSGALTSGVHTFPAVLQSSGLYSLSSVVTVPSSSLGTQTYICNVNHKPSNTKVDKKVEPKSCDKTHTCPPCPAPEAAGAPSVFLFPPKPKDTLMISRTPEVTCVVVDVSHEDPEVKFNWYVDGVEVHNAKTKPREEQYNSTYRVVSVLTVLHQDWLNGKEYKCKVSNKALPAPIEKTISKAKGQPREPQVYTLPPSRDELTKNQVSLTCLVKGFYPSDIAVEWESNGQPENNYKTTPPVLDSDGSFFLYSKLTVDKSRWQQGNVFSCSVMHEALHNHYTQKSLSLSPGK

SEQ ID NO: 71 - protein, 25 aa, Artificial Sequence [sequence omitted]

SEQ ID NO: 72 - protein, 17 aa, Artificial Sequence
  Synthetic Artificial Sequence
MSWVRQAPGKGLDWVAT

SEQ ID NO: 73 - protein, 38 aa, Artificial Sequence
  Synthetic Artificial Sequence
YYPDSVKGRFTISRDNSKNNLYLQMNSLRAEDTALYYC

SEQ ID NO: 74 - protein, 11 aa, Artificial Sequence
  Synthetic Artificial Sequence
WGQGTLVTVSS

SEQ ID NO: 75 - protein, 26 aa, Artificial Sequence
  Synthetic Artificial Sequence
DIQMTQSPSSMSASVGDRVTFTCRAS

SEQ ID NO: 76 - protein, 17 aa, Artificial Sequence
  Synthetic Artificial Sequence
LSWFQQKPGKSPKTLIY

SEQ ID NO: 77 - protein, 36 aa, Artificial Sequence
  Synthetic Artificial Sequence
RLVSGVPSRFSGSGSGQDYTLTISSLQPEDMATYYC

SEQ ID NO: 78 - protein, 10 aa, Artificial Sequence
  Synthetic Artificial Sequence
FGAGTKLELK

SEQ ID NO: 79 - protein, 20 aa, Artificial Sequence
  Synthetic Artificial Sequence
GGGGSGGGGSGGGGSGGGGS

SEQ ID NO: 80 - DNA, 60 bp, Artificial Sequence
  Synthetic Artificial Sequence
ggcggcggcggcagcggcggcggcggctccggaggaggcggctctggcggcggcggcagc

SEQ ID NO: 81 - protein, 15 aa, Artificial Sequence
  Synthetic Artificial Sequence
GGGGSGGGGSGGGGS

SEQ ID NO: 82 - DNA, 45 bp, Artificial Sequence
  Synthetic Artificial Sequence
ggcggcggcggctccggaggaggcggctctggcggcggcggcagc

SEQ ID NO: 83 - protein, 717 aa, Artificial Sequence
  Synthetic Artificial Sequence
QVQLVQSGAEVVKPGASVKVSCKASGYSFTGYTMNWVRQAPGQNLEWIGLINPYNAGTSYNQKFQGKVTLTVDKSTSTAYMELSSLRSEDTAVYYCARSEYRYGGDYFDYWGQGTTLTVSSASTKGPSVFPLAPSSKSTSGGTAALGCLVKDYFPEPVTVSWNSGALTSGVHTFPAVLQSSGLYSLSSVVTVPSSSLGTQTYICNVNHKPSNTKVDKKVEPKSCDKTHTCPPCPAPEAAGAPSVFLFPPKPKDTLMISRTPEVTCVVVDVSHEDPEVKFNWYVDGVEVHNAKTKPREEQYNSTYRVVSVLTVLHQDWLNGKEYKCKVSNKALPAPIEKTISKAKGQPREPQVYTLPPSRDELTKNQVSLTCLVKGFYPSDIAVEWESNGQPENNYKTTPPVLDSDGSFFLYSKLTVDKSRWQQGNVFSCSVMHEALHNHYTQKSLSLSPGKGGGGSGGGGSGGGGSGGGGSEVQLVESGGGLVQPGGSLRLSCAASGFAFSSYDMSWVRQAPGKGLDWVATISGGGRYTYYPDSVKGRFTISRDNSKNNLYLQMNSLRAEDTALYYCANRYGEAWFAYWGQGTLVTVSSGGGGSGGGGSGGGGSGGGGSDIQMTQSPSSMSASVGDRVTFTCRASQDINTYLSWFQQKPGKSPKTLIYRANRLVSGVPSRFSGSGSGQDYTLTISSLQPEDMATYYCLQYDEFPLTFGAGTKLELKR

SEQ ID NO: 84 - DNA, 2151 bp, Artificial Sequence
  Synthetic Artificial Sequence
caggtgcagctggtgcagtctggagcagaggtggtgaagccaggagcctctgtgaaggtgagctgtaaggccagcggctactccttcaccggctatacaatgaactgggtgaggcaggcaccaggacagaatctggagtggatcggcctgatcaacccttacaatgccggcacctcttataaccagaagtttcagggcaaggtgaccctgacagtggacaagtccacctctacagcctacatggagctgagctccctgcggagcgaggatacagccgtgtactattgcgcccggtccgagtacagatatggcggcgactactttgattattggggccagggcaccacactgaccgtgtctagcgcctccacaaaggggcccagcgtgtttcctctcgccccctcctccaaaagcaccagcggaggaaccgctgctctcggatgtctggtgaaggactacttccctgaacccgtcaccgtgagctggaatagcggcgctctgacaagcggagtccatacattccctgctgtgctgcaaagcagcggactctattccctgtccagcgtcgtcacagtgcccagcagcagcctgggcacccagacctacatctgtaacgtcaaccacaagccctccaacaccaaggtggacaagaaagtggagcccaaatcctgcgacaagacacacacctgtcccccctgtcctgctcccgaagctgctggagcccctagcgtcttcctctttcctcccaaacccaaggacaccctcatgatcagcagaacccctgaagtcacctgtgtcgtcgtggatgtcagccatgaggaccccgaggtgaaattcaactggtatgtcgatggcgtcgaggtgcacaacgccaaaaccaagcccagggaggaacagtacaactccacctacagggtggtgtccgtgctgacagtcctccaccaggactggctgaacggcaaggagtacaagtgcaaggtgtccaacaaggctctccctgcccccattgagaagaccatcagcaaggccaaaggccaacccagggagccccaggtctatacactgcctccctccagggacgaactcaccaagaaccaggtgtccctgacctgcctggtcaagggcttttatcccagcgacatcgccgtcgagtgggagtccaacggacagcccgagaataactacaagaccacccctcctgtcctcgactccgacggctccttcttcctgtacagcaaactgaccgtcgataaatctaggtggcagcagggcaacgtgttctcttgttccgtgatgcatgaagcactgcacaaccattatacccagaagtctctgagcctgtcccccggcaagggcggcggcggctctggaggaggaggcagcggcggaggaggctccggaggcggcggctctgaggtgcagctggtggagtctggaggaggactggtgcagcctggaggctccctgaggctgtcttgcgcagcaagcggattcgcctttagctcctacgacatgagctgggtgcggcaggcacctggcaagggtctggattgggtggcaaccatcagcggaggcggcagatacacatactatcccgactccgtgaagggcaggttcaccatctcccgcgataactctaagaacaatctgtatctgcagatgaacagcctgagggccgaggacacagccctgtactattgcgccaaccgctacggcgaggcctggtttgcctattggggccagggcaccctggtgacagtgtctagcggcggcggcggcagcggcggcggcggctccggaggaggcggctctggcggcggcggcagcgatatccagatgacccagtccccctcctctatgtctgccagcgtgggcgaccgggtgaccttcacatgtagagcctcccaggatatcaacacctacctgtcttggtttcagcagaagcccggcaagagccctaagacactgatctatcgggccaatagactggtgagcggagtgccttcccggttctccggctctggcagcggacaggactataccctgacaatcagctccctgcagccagaggatatggccacatactattgcctgcagtatgacgagttccccctgaccttcggggctggcactaagctggagctgaaaaga

SEQ ID NO: 85 - protein, 712 aa, Artificial Sequence
  Synthetic Artificial Sequence
QVQLVQSGAEVVKPGASVKVSCKASGYSFTGYTMNWVRQAPGQNLEWIGLINPYNAGTSYNQKFQGKVTLTVDKSTSTAYMELSSLRSEDTAVYYCARSEYRYGGDYFDYWGQGTTLTVSSASTKGPSVFPLAPSSKSTSGGTAALGCLVKDYFPEPVTVSWNSGALTSGVHTFPAVLQSSGLYSLSSVVTVPSSSLGTQTYICNVNHKPSNTKVDKKVEPKSCDKTHTCPPCPAPEAAGAPSVFLFPPKPKDTLMISRTPEVTCVVVDVSHEDPEVKFNWYVDGVEVHNAKTKPREEQYNSTYRVVSVLTVLHQDWLNGKEYKCKVSNKALPAPIEKTISKAKGQPREPQVYTLPPSRDELTKNQVSLTCLVKGFYPSDIAVEWESNGQPENNYKTTPPVLDSDGSFFLYSKLTVDKSRWQQGNVFSCSVMHEALHNHYTQKSLSLSPGKGGGGSGGGGSGGGGSGGGGSEVQLVESGGGLVQPGGSLRLSCAASGFAFSSYDMSWVRQAPGKGLDWVATISGGGRYTYYPDSVKGRFTISRDNSKNNLYLQMNSLRAEDTALYYCANRYGEAWFAYWGQGTLVTVSSGGGGSGGGGSGGGGSDIQMTQSPSSMSASVGDRVTFTCRASQDINTYLSWFQQKPGKSPKTLIYRANRLVSGVPSRFSGSGSGQDYTLTISSLQPEDMATYYCLQYDEFPLTFGAGTKLELKR

SEQ ID NO: 86 - DNA, 2148 bp, Artificial Sequence
  Synthetic Artificial Sequence
caggtgcagctggtgcagtctggagcagaggtggtgaagccaggagcctctgtgaaggtgagctgtaaggccagcggctactccttcaccggctatacaatgaactgggtgaggcaggcaccaggacagaatctggagtggatcggcctgatcaacccttacaatgccggcacctcttataaccagaagtttcagggcaaggtgaccctgacagtggacaagtccacctctacagcctacatggagctgagctccctgcggagcgaggatacagccgtgtactattgcgcccggtccgagtacagatatggcggcgactactttgattattggggccagggcaccacactgaccgtgtctagcgcctccacaaaggggcccagcgtgtttcctctcgccccctcctccaaaagcaccagcggaggaaccgctgctctcggatgtctggtgaaggactacttccctgaacccgtcaccgtgagctggaatagcggcgctctgacaagcggagtccatacattccctgctgtgctgcaaagcagcggactctattccctgtccagcgtcgtcacagtgcccagcagcagcctgggcacccagacctacatctgtaacgtcaaccacaagccctccaacaccaaggtggacaagaaagtggagcccaaatcctgcgacaagacacacacctgtcccccctgtcctgctcccgaagctgctggagcccctagcgtcttcctctttcctcccaaacccaaggacaccctcatgatcagcagaacccctgaagtcacctgtgtcgtcgtggatgtcagccatgaggaccccgaggtgaaattcaactggtatgtcgatggcgtcgaggtgcacaacgccaaaaccaagcccagggaggaacagtacaactccacctacagggtggtgtccgtgctgacagtcctccaccaggactggctgaacggcaaggagtacaagtgcaaggtgtccaacaaggctctccctgcccccattgagaagaccatcagcaaggccaaaggccaacccagggagccccaggtctatacactgcctccctccagggacgaactcaccaagaaccaggtgtccctgacctgcctggtcaagggcttttatcccagcgacatcgccgtcgagtgggagtccaacggacagcccgagaataactacaagaccacccctcctgtcctcgactccgacggctccttcttcctgtacagcaaactgaccgtcgataaatctaggtggcagcagggcaacgtgttctcttgttccgtgatgcatgaagcactgcacaaccattatacccagaagtctctgagcctgtcccccggcaagggcggcggcggctctggaggaggaggcagcggcggaggaggctccggaggcggcggctctgaggtgcagctggtggagtctggaggaggactggtgcagcctggaggctccctgaggctgtcttgcgcagcaagcggattcgcctttagctcctacgacatgagctgggtgcggcaggcacctggcaagggtctggattgggtggcaaccatcagcggaggcggcagatacacatactatcccgactccgtgaagggcaggttcaccatctcccgcgataactctaagaacaatctgtatctgcagatgaacagcctgagggccgaggacacagccctgtactattgcgccaaccgctacggcgaggcctggtttgcctattggggccagggcaccctggtgacagtgtctagcggcggcggcggctccggaggaggcggctctggcggcggcggcagcgatatccagatgacccagtccccctcctctatgtctgccagcgtgggcgaccgggtgaccttcacatgtagagcctcccaggatatcaacacctacctgtcttggtttcagcagaagcccggcaagagccctaagacactgatctatcgggccaatagactggtgagcggagtgccttcccggttctccggctctggcagcggacaggactataccctgacaatcagctccctgcagccagaggatatggccacatactattgcctgcagtatgacgagttccccctgaccttcggggctggcactaagctggagctgaaaagatgataagaattc

SEQ ID NO: 87 - protein, 558 aa, Artificial Sequence
  Synthetic Artificial Sequence
MCPRAARAPATLLLALGAVLWPAAGAWELTILHTNDVHSRLEQTSEDSSKCVNASRCMGGVARLFTKVQQIRRAEPNVLLLDAGDQYQGTIWFTVYKGAEVAHFMNALRYDAMALGNHEFDNGVEGLIEPLLKEAKFPILSANIKAKGPLASQISGLYLPYKVLPVGDEVVGIVGYTSKETPFLSNPGTNLVFEDEITALQPEVDKLKTLNVNKIIALGHSGFEMDKLIAQKVRGVDVVVGGHSNTFLYTGNPPSKEVPAGKYPFIVTSDDGRKVPVVQAYAFGKYLGYLKIEFDERGNVISSHGNPILLNSSIPEDPSIKADINKWRIKLDNYSTQELGKTIVYLDGSSQSCRFRECNMGNLICDAMINNNLRHTDEMFWNHVSMCILNGGGIRSPIDERNNGTITWENLAAVLPFGGTFDLVQLKGSTLKKAFEHSVHRYGQSTGEFLQVGGIHVVYDLSRKPGDRVVKLDVLCTKCRVPSYDPLKMDEVYKVILPNFLANGGDGFQMIKDELLRHDSGDQDINVVSTYISKMKVIYPAVEGRIKFSTGSHHHHHH

SEQ ID NO: 88 - DNA, 1674 bp, Artificial Sequence
  Synthetic Artificial Sequence
atgtgtcctagagccgccagagctccagctacactgctgctggctctgggagcagtcctctggccagcagcaggagcttgggaactgaccatcctgcacaccaacgacgtgcacagcaggctggaacagaccagcgaggacagcagcaagtgcgtgaacgccagtcgctgtatgggaggagtggcaaggctgttcaccaaggtgcagcagatccggagagccgaacctaacgtgctgctgctggacgccggagatcagtatcagggaaccatctggttcaccgtgtacaagggcgccgaagtggcccacttcatgaacgctctgcgctacgacgctatggccctgggcaatcacgagttcgataacggcgtggagggactgatcgagcctctgctgaaggaggccaagttccccatcctgagcgccaacatcaaggccaagggacctctggctagccagattagcggcctgtacctgccttacaaggtgctgcccgtgggagacgaagtggtgggaatcgtgggctacaccagcaaggagacccctttcctgagcaacccaggcaccaacctggtgttcgaggacgagatcaccgctctgcagccagaggtggacaagctgaagaccctgaacgtgaacaagatcatcgccctgggacacagcggcttcgagatggacaagctgatcgcccagaaagtgcgaggagtggacgtggtcgtgggcggacacagcaacaccttcctgtacaccggcaaccctccttctaaggaagtgccagccggcaagtaccccttcatcgtgaccagcgacgacggaagaaaggtgccagtggtgcaggcttacgccttcggcaagtacctgggctacctgaagatcgagttcgacgagcggggcaacgtgatctctagccacggcaaccccatcctgctgaacagcagcatcccagaggaccccagcatcaaggccgacatcaacaagtggcggatcaagctggacaactacagcacccaggagctgggaaagaccatcgtgtacctggacggcagctctcagtcttgccggttccgcgagtgcaacatgggcaacctgatttgcgacgccatgatcaacaacaacctgcggcacaccgacgagatgttttggaaccacgtcagcatgtgcatcctgaacggcggaggcatcagaagccctattgacgagcggaacaacggcaccatcacttgggagaacctggcagcagtgctgccttttggcggaacattcgacctggtgcagctgaagggcagcacactgaagaaggccttcgagcacagcgtgcacagatacggccagagcacaggcgagttcctgcaggtcggaggaatccacgtggtgtacgacctgagcaggaagccaggagacagagtggtgaagctggacgtgctctgcaccaagtgtcgggtgccaagctacgaccccctgaagatggacgaggtgtacaaggtcatcctgcccaacttcctggctaacggaggagacggcttccagatgatcaaggacgagctgctgaggcacgacagcggagaccaggacatcaacgtcgtgtccacctacatcagcaagatgaaggtcatctaccccgccgtggaaggcaggatcaagttcagcaccggctctcaccaccaccatcaccac

SEQ ID NO: 89 - protein, 232 aa, Artificial Sequence
  Synthetic Artificial Sequence
PRGPTIKPCPPCKCPAPNLLGGPSVFIFPPKIKDVLMISLSPIVTCVVVDVSEDDPDVQISWFVNNVEVHTAQTQTHREDYNSTLRVVSALPIQHQDWMSGKEFKCKVNNKDLPAPIERTISKPKGSVRAPQVYVLPPPEEEMTKKQVTLTCMVTDFMPEDIYVEWTNNGKTELNYKNTEPVLDSDGSYFMYSKLRVEKKNWVERNSYSCSVVHEGLHNHHTTKSFSRTPGK

SEQ ID NO: 90 - protein, 249 aa, Artificial Sequence
  Synthetic Artificial Sequence
QVQLQQSGAEVVKPGASMKMSCKASGYSFTGYTMNWVKQAHGQNLEWIGLINPYNAGTSYNQKFQGKATLTVDKSTSTAYMELSSLRSEDTAVYYCARSEYRYGGDYFDYWGQGTTLTVSSGGGGSGGGGSGGGGSDIVMTQSPSSLAVSVGERVTISCKSSQSLLNSSNQKNYLAWYQQKPGQAPKLLIYFASTRESGVPDRFSGSGSGTDFTLTISSVQAEDVADYYCQQHYDTPYTFGGGTKLEIK

SEQ ID NO: 91 - DNA, 837 bp, Artificial Sequence
  Synthetic Artificial Sequence
caggtgcagctgcagcagtctggagcagaggtggtgaagccaggagcctctatgaagatgagctgtaaggccagcggctactccttcaccggctatacaatgaactgggtgaagcaggcccacggccagaatctggagtggatcggcctgatcaacccttacaatgccggcacctcttataaccagaagtttcagggcaaggccaccctgacagtggacaagtccacctctacagcctacatggagctgagctccctgcggagcgaggatacagccgtgtactattgcgcccggtccgagtacagatatggcggcgactactttgattattggggccagggcaccacactgaccgtgtctagcggcctgtacggcctgtacggcctgtacggcctgtacagcgagaggggcctgtacggcctgtacggcctgtacggcctgtacagcgagaggggcctgtacggcctgtacggcctgtacggcctgtacagcgagagggacatcgtgatgacccagtccccaagctccctggccgtgtctgtgggagagcgggtgacaatctcctgtaagtctagccagtctctgctgaactcctctaatcagaagaactacctggcctggtatcagcagaagcccggccaggcccctaagctgctgatctacttcgcctctaccagggagagcggagtgccagacagattctctggcagcggctccggcacagacttcaccctgacaatcagctccgtgcaggcagaggacgtggcagattactattgccagcagcactacgataccccctatacatttggcggcggcaccaagctggagatcaag

SEQ ID NO: 92 - DNA, 363 bp, Artificial Sequence
  Synthetic Artificial Sequence
caggtgcagctgcagcagtctggagcagaggtggtgaagccaggagcctctatgaagatgagctgtaaggccagcggctactccttcaccggctatacaatgaactgggtgaagcaggcccacggccagaatctggagtggatcggcctgatcaacccttacaatgccggcacctcttataaccagaagtttcagggcaaggccaccctgacagtggacaagtccacctctacagcctacatggagctgagctccctgcggagcgaggatacagccgtgtactattgcgcccggtccgagtacagatatggcggcgactactttgattattggggccagggcaccacactgaccgtgtctagc

SEQ ID NO: 93 - protein, 121 aa, Artificial Sequence
  Synthetic Artificial Sequence
QVQLQQSGAEVVKPGASMKMSCKASGYSFTGYTMNWVKQAHGQNLEWIGLINPYNAGTSYNQKFQGKATLTVDKSTSTAYMELSSLRSEDTAVYYCARSEYRYGGDYFDYWGQGTTLTVSS

SEQ ID NO: 94 - DNA, 339 bp, Artificial Sequence
  Synthetic Artificial Sequence
gacatcgtgatgacccagtccccaagctccctggcaatgtctgtgggagagagggtgacaatgtcctgtaagtctagccagtctctgctgaactcctctaatcagaagaactacctggcctggtatcagcagaagcccggccaggcccctaagctgctggtgtactttgcctctaccagggagagcggagtgccagacagattctctggcagcggctccggcacagacttcaccctgacaatcagctccgtgcaggcagaggacctggcagattatttctgccagcagcactacgataccccctatacatttggcggcggcaccaagctggagatcaag

SEQ ID NO: 95 - protein, 113 aa, Artificial Sequence
  Synthetic Artificial Sequence
DIVMTQSPSSLAMSVGERVTMSCKSSQSLLNSSNQKNYLAWYQQKPGQAPKLLVYFASTRESGVPDRFSGSGSGTDFTLTISSVQAEDLADYFCQQHYDTPYTFGGGTKLEIK

SEQ ID NO: 96 - protein, 220 aa, Artificial Sequence
  Synthetic Artificial Sequence
DIVMTQSPSSLAVSVGERVTISCKSSQSLLNSSNQKNYLAWYQQKPGQAPKLLIYFASTRESGVPDRFSGSGSGTDFTLTISSVQAEDVADYYCQQHYDTPYTFGGGTKLEIKRTVAAPSVFIFPPSDEQLKSGTASVVCLLNNFYPREAKVQWKVDNALQSGNSQESVTEQDSKDSTYSLSSTLTLSKADYEKHKVYACEVTHQGLSSPVTKSFNRGEC

SEQ ID NO: 97 - protein, 121 aa, Artificial Sequence; identical to SEQ ID NO: 20
  Synthetic Artificial Sequence

SEQ ID NO: 98 - protein, 113 aa, Artificial Sequence; identical to SEQ ID NO: 22
  Synthetic Artificial Sequence

SEQ ID NO: 99 - protein, 113 aa, Artificial Sequence; identical to SEQ ID NO: 24
  Synthetic Artificial Sequence

SEQ ID NO: 100 - DNA, 660 bp, Artificial Sequence
  Synthetic Artificial Sequence
gacatcgtgatgacccagtccccaagctccctggccgtgtctgtgggagagcgggtgacaatctcctgtaagtctagccagtctctgctgaactcctctaatcagaagaactacctggcctggtatcagcagaagcccggccaggcccctaagctgctgatctacttcgcctctaccagggagagcggagtgccagacagattctctggcagcggctccggcacagacttcaccctgacaatcagctccgtgcaggcagaggacgtggcagattactattgccagcagcactacgataccccctatacatttggcggcggcaccaagctggagatcaagcgtacggtggcagccccatctgtcttcatttttccccctagtgacgagcagctgaaatccggaacagcctctgtggtctgtctgctgaacaatttctaccctcgcgaagccaaggtgcagtggaaagtcgataacgctctgcagagtggcaattcacaggagagcgtgactgaacaggactccaaggattctacctatagtctgagctccactctgaccctgtccaaagcagattacgaaaagcacaaagtgtatgcctgtgaggtcacccaccaggggctgagttctccagtcaccaaatccttcaacagaggcgaatgt